European Patent Application EP 4 728 866 A1, published April 22, 2026. Title: Agent for controlling plant parasitic nematode. Applicant: NATIONAL UNIVERSITY CORPORATION KUMAMOTO UNIVERSITY. Application JP. The sequence listing filed with the application follows.

SEQUENCE LISTING (16 sequences)

SEQ ID NO: 1 - protein, 1060 aa, Oryza sativa
MPIGAISTVGPAISPGIKIAEIAESFVARKYRRLRDYRKDVAQLVGEVGKIAVAVDTVEEQEQFMSDRRIVGQLSELMDAIHEAEDILDAVDYRDSIWARKHKVRQVIHSIVEQAKRIVGIDGALNRLDKSMNDLPRMQQNQRDLVQLSNFRSSQGGGDGGASASRPRSATGLLPDGKLYGYKEEYDRLVSALLYDPPRRPGGNGNGGGQVVAVVGDGGVGKTALAQHALRHVDVQARFDHVIWASVPHKYRNKDLLAEIWMSGPGATATATATHRCADQMSFGALQAEFVRLVSLSSQRYLLVLDDVCNDESDDDDHQRSRKEWEDVLAPFKQGERGNRILVTTRASICCATLNAGTRIQLNGIAADELLLLLKKSAFGDHDKKHAPHLDEVLTSLAEKLKDCPSAAAVVAARVRNKARRKDWEEALALLDAGRVLSPRRHESRYREFRDLPHHLQSCLHFCSLFPNNWMFHPDKLVRMWIAHGIIVVGDAHAHAPIDGRSMEEEEQVGRRYIRDLVSRSFFHLQPAKNGSRTMYLAIRQHVHSMLLSVSASYFFRVTSSSLGRRIPPTVRHLSVAPVTVTDQDQGQGGCLDLDWLKKHPVLNKLRTLLVFDGRMSAMDGDILRQLEAVRVLDLTSTNITADFPKGIGKLKHLRYLGLPKSLKKLPEGVNKLLHLQALVSAEDKLQGSVELCADSGCRKPGHGLEALAHMNSLCGELSIKGLQAVSNREEAHRAHLERKEFLKALKLEWEPSLQLQEPSESSHEQVLEGLKPPCKIEELHIRQYLGRTSPSWLESNLLSGLRYLYLRNCRNWQVLPTLSQLPHLKVICIKEMCSVQRIDHRLYGGDGVFKSLETLILDDMPNLVEWAAEATDEKFPHLQKISMLNCPKLEKLPRVPRTVRNMEIQKHPSCYLHLSPSSSSSSSISFTLDIRADAVHLLHEDFLHPDHIKAIGSIRIEHYTWSTEPNLNLLASVRSLSLTRCPVTDRSLSMCLHKLQSLERLEISDCPELHDFPDDAMPMMASLKSLEFNGCHPLLMKKLQGRTGAAWERIRSIQRLEIV

SEQ ID NO: 2 - DNA, 3183 bp, Oryza sativa
  source 1..3183: mol_type = unassigned DNA
atgccgattggagcaatttcgacggttgggccggcgatttcgccgggcatcaagatcgccgaaatcgcggaatcctttgtggcgaggaagtacagacgcttgagagattacagaaaggacgttgcacagctggtgggtgaagtggggaagatcgcagtggccgtggacacggtggaggaacaggaacagttcatgagcgaccgtcggatcgtggggcaactgagtgagctgatggacgccatccacgaggctgaggacatcttggacgccgtcgactacagagacagtatctgggcgaggaagcacaaggtcaggcaggttatccattctatagttgaacaagctaagcggatagtcggaatagacggcgcgttgaaccggctggacaagtcgatgaatgacctgccacggatgcagcagaaccagcgggatcttgtccagctgtcaaatttccggtcatcacaaggaggaggagatgggggtgcgtccgcgtcgaggccaagatcggccacgggcctattgccggacggcaaactctacggttacaaggaggagtacgatcggctggtgtcggccttgctgtacgatcctccccggcggcctggtggcaatggcaatggcggcggtcaagtcgtggcggtcgtcggcgacggcggcgttggcaagactgcgcttgctcagcacgcgctgaggcacgtggacgttcaagcaaggtttgatcatgtgatctgggcgagcgtcccacacaagtacaggaacaaggacctcttggctgagatctggatgtccggaccgggtgctactgctactgctactgctacacacaggtgcgccgaccagatgagctttggtgcccttcaggcggagttcgtcaggctggtgtcactgtcatcccagaggtacctgctcgtcctcgacgatgtctgcaacgatgagtcggacgacgacgatcatcagcggagcaggaaggaatgggaggatgtccttgcccccttcaaacaaggggaacgagggaacaggatcctggtgacaacccgtgcaagcatctgttgcgccacgctcaacgcaggcaccaggatccagctaaacgggatcgccgccgacgagctcttgcttctgctcaagaagagcgcgttcggcgaccacgacaagaagcatgccccacacctggacgaggttttgacgagcctcgcggagaagctcaaggactgcccatcagcagcagccgtcgttgctgccagggtgaggaacaaggccagaaggaaagactgggaggaagccttggccctcctggatgcaggccgcgttctctcaccgcgtcgccatgaatccagataccgcgaattccgcgatctgccgcaccacctccagagctgcttgcacttctgcagcttgttccccaacaactggatgtttcatcctgacaagttggtcagaatgtggatagcacatggcatcatcgtcgtcggcgatgcgcatgcgcatgcgccgattgatgggagaagcatggaggaagaagaacaagtgggaagacgctatatcagggacctggtgtcaagatccttcttccatctccaacctgcaaagaatggcagcagaaccatgtatctcgccattcgtcagcacgtccattcgatgctgctctccgtctccgctagctatttcttcagggttactagcagtagcttgggaagaagaatccctcctaccgttcgccacctgtctgtagctcctgtgacagtgacagatcaggatcagggacaaggtggttgccttgacctggactggctcaagaaacaccccgtgctgaacaagttgcggacattgttggttttcgatggacgaatgagcgccatggacggcgacatactcagacagctggaggccgtcagggtgctggacctcacctccacaaacatcaccgcagatttccccaaaggcatcggtaagctgaagcatctgaggtacctaggccttcccaaatcgctcaagaaacttcctgaaggagtcaacaagctactgcatctccaagcactggtttcagccgaggacaaactacagggatcagttgagctctgcgctgacagtggctgcaggaagccggggcatggcctggaagcgctcgcacacatgaactctctctgcggtgaactgagcataaaggggctccaagctgtctccaacagagaggaagcacacagggctcaccttgagaggaaagagtttctcaaggccctcaagttggagtgggagccttcattacaactacaggaaccctcagaatcgtcacatgagcaagttctcgagggactcaagccaccctgcaagatcgaagagttgcacatcagacagtacctgggcagaacatcgcctagttggttggagagcaatctgctgtcaggtttgagatacctgtatctcagaaactgcaggaattggcaggtcctgccgaccctgagccagctacctcatctcaaggttatctgtatcaaagagatgtgctctgtccagcggattgaccataggctttacggcggcgacggcgttttcaagtcactggagacacttatcctggatgatatgccaaatttggtcgagtgggcggctgaagcaactgacgaaaaattccctcatcttcagaagatatccatgttgaactgccccaaactggagaagctaccccgggtgccacgcaccgtcaggaacatggagatacaaaaacacccttcttgttacctccatctttcaccttcatcatcgtcatcgtcatcgatttcttttaccttggatatccgtgcggatgctgtccatctgctgcatgaagatttcctgcatccggatcacataaaggcaatcggttcaatcagaatcgagcactacacatggtcgactgagccaaacctcaacctccttgcttctgttaggagcctgtcgttaacccgatgtcctgtgacagacaggagtttgagcatgtgcctgcataaactgcagtccctcgagagactagagatatctgattgccctgaacttcatgacttccccgatgatgccatgcctatgatggcatccttgaaatccctcgagtttaacggatgccatcctcttcttatgaagaagctacaaggcaggactggcgctgcctgggaaaggattcgctccatccagcgactagaaatcgtttaa

SEQ ID NO: 3 - DNA, 1020 bp, Oryza sativa
  source 1..1020: mol_type = unassigned DNA
atgccgattggagcaatttcgacggttgggccggcgatttcgccgggcatcaagatcgccgaaatcgcggaatcctttgtggcgaggaagtacagacgcttgagagattacagaaaggacgttgcacagctggtgggtgaagtggggaagatcgcagtggccgtggacacggtggaggaacaggaacagttcatgagcgaccgtcggatcgtggggcaactgagtgagctgatggacgccatccacgaggctgaggacatcttggacgccgtcgactacagagacagtatctgggcgaggaagcacaaggtcaggcaggttatccattctatagttgaacaagctaagcggatagtcggaatagacggcgcgttgaaccggctggacaagtcgatgaatgacctgccacggatgcagcagaaccagcgggatcttgtccagctgtcaaatttccggtcatcacaaggaggaggagatgggggtgcgtccgcgtcgaggccaagatcggccacgggcctattgccggacggcaaactctacggttacaaggaggagtacgatcggctggtgtcggccttgctgtacgatcctccccggcggcctggtggcaatggcaatggcggcggtcaagtcgtggcggtcgtcggcgacggcggcgttggcaagactgcgcttgctcagcacgcgctgaggcacgtggacgttcaagcaaggtttgatcatgtgatctgggcgagcgtcccacacaagtacaggaacaaggacctcttggctgagatctggatgtccggaccgggtgctactgctactgcggctacacacaggtgcgccgaccagatgagctttggtgcccttcaggcggagttcgtcaggctggtgtctctgtcatcccagaggtacctgctcgtcctcgacgatgtctgcaacgatgagtcggacgacgacgatcatcagcggagcaggaaggaatgggaggatgtccttgcccccttcaaacaaggggaacgagggaacacatga

SEQ ID NO: 4 - DNA, 1020 bp, Oryza sativa; identical to SEQ ID NO: 3
  source 1..1020: mol_type = unassigned DNA

SEQ ID NO: 5 - DNA, 687 bp, Oryza sativa
  source 1..687: mol_type = unassigned DNA
atgccgattggagcaatttcgacggttgggccggcgatttcgccgggcatcaagatcgccgaaatcgcggaatcctttgtggcgaggaagtacagacgcttgagagattacagaaaggacgttgcacagctggtgggtgaagtggggaagatcgcagtggccgtggacacggtggaggaacaggaacagttcatgagcgaccgtcggatcgtggggcaactgagtgagctgatggacgccatccacgaggctgaggacatcttggacgccgtcgactacagagacagtatctgggcgaggaagcacaaggtcaggcaggttatccattctatagttgaacaagctaagcggatagtcggaatagacggcgcgttgaaccggctggacaagtcgatgaatgacctgccacggatgcagcagaaccagcgggatcttgtccagctgtcaaatttccggtcatcacaaggaggaggagatgggggtgcgtccgcgtcgaggccaagatcggccacgggcctattgccggacggcaaactctatacaaggaggagtacgatcggctggtgtcggccttgctatacgatcctccccggcggcctggtggcaatggcaatggcggcggtcaagtcgtggcggtcgtcggcgacggcggcgttggcaagactgcgcttgctcagcacgcgctga

SEQ ID NO: 6 - DNA, 687 bp, Oryza sativa; identical to SEQ ID NO: 5
  source 1..687: mol_type = unassigned DNA

SEQ ID NO: 7 - DNA, 3183 bp, Oryza sativa
  source 1..3183: mol_type = unassigned DNA
atgccgattggagcaatttcgacggttgggccggcgatttcgccgggcatcaagatcgccgaaatcgcggaatcctttgtggcgaggaagtacagacgcttgagagattacagaaaggacgttgcacagctggtgggtgaagtggggaagatcgcagtggccgtggacacggtggaggaacaggaacagttcatgagcgaccgtcggatcgtggggcaactgagtgagctgatggacgccatccacgaggctgaggacatcttggacgccgtcgactacagagacagtatctgggcgaggaagcacaaggtcaggcaggttatccattctatagttgaacaagctaagcggatagtcggaatagacggcgcgttgaaccggctggacaagtcgatgaatgacctgccacggatgcagcagaaccagcgggatcttgtccagctgtcgaatttccggtcatcacaaggaggaggagatgggggtgcgtccgcgtcgaggccaagatcggccacgggcctattgccggacggcaaactctacggttacaaggaggagtacgatcggctggtgtcggccttgctgtacgatcctccccggcggcctggtggcaatggcaatggcggcggtcaagtcgtggcggtcgtcggcgacggcggcgttggcaagactgcgcttgctcagcacgcgctgaggcacgtggacgttcaagcaaggtttgatcatgtgatatgggcgagtgtcccacacaagtacaggaacaaggacctcttggctgagatctggatgtccggaccgggtgctactgctactgctactgctacacacaggtgcgccgaccagatgagctttggtgcccttcaggcggagttcgtcaggctggtgtcactgtcatcccagaggtacctgctcgtcctcgacgatgtctgcaacgatgagtcggacggcgacgatcatcagcggagtaggaaggaatgggaggatgtccttgcccccttcaaacaaggggaacgagggaacaggatcctggtgacaacccgtgcaagcatctgttgcgccacgctcaacgcaggcaccaggatccagctaaacgggatcgccgccgacgagctcttgcttctgctcaagaagagcgcgttcggcgaccacgacaagaagcatgccccacacctggacgaggttttgacgagcctcgcggagaagctcaaggactgcccatcagcagcagccgtcgttgctgccagggtgaggaacaaggccagaaggaaagactgggaggaagccttggccctcctggatgcaggccgcgttctctcaccgcgtcgccatgaatccagataccgcgaattccgcgatctgccgcaccacctccagagctgcttgcacttctgcagcttgttccccaacaactggatgtttcatcctgacaagttggtcagaatgtggatagcacatggcatcatcgtcgtcggcgatgcgcatgcgcatgcgccgattgatgggagaagcatggaggatgaagaacaagtgggaagacgctatatcagggacctggtgtcaagatccttcttccatctccaacctgcaaagaatggcagcagaaccatgtatctcgccattcgtcagcacgtccattcgatgctgctctccgtctccgctagctatttcttcagggttactagcagtagcttgggaagaagaatccctcctaccgttcgccacctgtctgtagctcctgtgacagtgacagatcaggatcagggacaaggtggttgccttgacctggactggctcaagaaacaccccgtgctgaacaagttgcggacattgttggttttcgatggacgaatgagcgccatggacggcgacatactcagacagctggaggccgtcagggtgctggacctcacctccacaaacatcaccgcagatttccccaaaggcatcggtaagctgaagcatctgaggtacctaggccttcccaaatcgctcaagaaacttcctgaaggagtcaacaagctactgcatctccaagcactggtttcagccgaggacaaactacagggatcagttgagctctgcgctgacagtggctgcaggaagccggggcatggcctggaagcgctcgcacacatgaactctctctgcggtgaactcagcataaaggggctccaagctgtctccaacagagaggaagcacacagggctcaccttgagaggaaagagtttctcaaggtcctcaagttggagtgggagccttcattacaactacaagaaccctcagaatcgtcacatgagcaagttctcgagggactcaagccaccctgcaagatcgaagagttgcacatcagacagtacctgggcagaacatcgcctagttggttggagagcaatctgctgtcaggtttgagatacctgtatctcagaaactgcaggaattggcaggtcctgccgaccctgagccagctacctcatctcaaggttatctgtatcaaagagatgtgctctgtccagcggattgaccataggctttacggcggcgacggcgttttcaagtcactggagacacttatcctggatgatatgccaaatttggtcgagtgggcggctgaagcaactgacgaaaaattccctcatcttcagaagatatccatgttgaactgccccaaactggagaagctaccccgggtgccacgcaccgtcaggaacatggagatacaaaaacacccttcttgttacctccatctttcaccttcatcatcgtcatcgtcatcgatttcttttaccttggatatccgtgcggatgctgtccatctgctgcatgaagatttcctgcatccggatcacataaaggcaatcggttcaatcagaatcgagcactacacatggtcgactgagccaaacctcaacctccttgcttctgttaggagcctgtcgttaacccgatgtcctgtgacagacaggagtttgagcatgtgcctgcataaactgcagtccctcgagagactagagatatctgattgccctgaacttcatgacttccccgatgatgccatgcctatgatggcatccttgaaatccctcgagtttaacggatgccatcctcttcttatgaagaagcaacaaggcaggactggcgctgcctgggaaaggattcgctccatccagcgactagaaatcgtttaa

SEQ ID NO: 8 - protein, 339 aa, Oryza sativa
MPIGAISTVGPAISPGIKIAEIAESFVARKYRRLRDYRKDVAQLVGEVGKIAVAVDTVEEQEQFMSDRRIVGQLSELMDAIHEAEDILDAVDYRDSIWARKHKVRQVIHSIVEQAKRIVGIDGALNRLDKSMNDLPRMQQNQRDLVQLSNFRSSQGGGDGGASASRPRSATGLLPDGKLYGYKEEYDRLVSALLYDPPRRPGGNGNGGGQVVAVVGDGGVGKTALAQHALRHVDVQARFDHVIWASVPHKYRNKDLLAEIWMSGPGATATAATHRCADQMSFGALQAEFVRLVSLSSQRYLLVLDDVCNDESDDDDHQRSRKEWEDVLAPFKQGERGNT

SEQ ID NO: 9 - protein, 339 aa, Oryza sativa; identical to SEQ ID NO: 8

SEQ ID NO: 10 - protein, 228 aa, Oryza sativa
MPIGAISTVGPAISPGIKIAEIAESFVARKYRRLRDYRKDVAQLVGEVGKIAVAVDTVEEQEQFMSDRRIVGQLSELMDAIHEAEDILDAVDYRDSIWARKHKVRQVIHSIVEQAKRIVGIDGALNRLDKSMNDLPRMQQNQRDLVQLSNFRSSQGGGDGGASASRPRSATGLLPDGKLYTRRSTIGWCRPCYTILPGGLVAMAMAAVKSWRSSATAALARLRLLSTR

SEQ ID NO: 11 - protein, 228 aa, Oryza sativa; identical to SEQ ID NO: 10

SEQ ID NO: 12 - protein, 1060 aa, Oryza sativa
MPIGAISTVGPAISPGIKIAEIAESFVARKYRRLRDYRKDVAQLVGEVGKIAVAVDTVEEQEQFMSDRRIVGQLSELMDAIHEAEDILDAVDYRDSIWARKHKVRQVIHSIVEQAKRIVGIDGALNRLDKSMNDLPRMQQNQRDLVQLSNFRSSQGGGDGGASASRPRSATGLLPDGKLYGYKEEYDRLVSALLYDPPRRPGGNGNGGGQVVAVVGDGGVGKTALAQHALRHVDVQARFDHVIWASVPHKYRNKDLLAEIWMSGPGATATATATHRCADQMSFGALQAEFVRLVSLSSQRYLLVLDDVCNDESDGDDHQRSRKEWEDVLAPFKQGERGNRILVTTRASICCATLNAGTRIQLNGIAADELLLLLKKSAFGDHDKKHAPHLDEVLTSLAEKLKDCPSAAAVVAARVRNKARRKDWEEALALLDAGRVLSPRRHESRYREFRDLPHHLQSCLHFCSLFPNNWMFHPDKLVRMWIAHGIIVVGDAHAHAPIDGRSMEDEEQVGRRYIRDLVSRSFFHLQPAKNGSRTMYLAIRQHVHSMLLSVSASYFFRVTSSSLGRRIPPTVRHLSVAPVTVTDQDQGQGGCLDLDWLKKHPVLNKLRTLLVFDGRMSAMDGDILRQLEAVRVLDLTSTNITADFPKGIGKLKHLRYLGLPKSLKKLPEGVNKLLHLQALVSAEDKLQGSVELCADSGCRKPGHGLEALAHMNSLCGELSIKGLQAVSNREEAHRAHLERKEFLKVLKLEWEPSLQLQEPSESSHEQVLEGLKPPCKIEELHIRQYLGRTSPSWLESNLLSGLRYLYLRNCRNWQVLPTLSQLPHLKVICIKEMCSVQRIDHRLYGGDGVFKSLETLILDDMPNLVEWAAEATDEKFPHLQKISMLNCPKLEKLPRVPRTVRNMEIQKHPSCYLHLSPSSSSSSSISFTLDIRADAVHLLHEDFLHPDHIKAIGSIRIEHYTWSTEPNLNLLASVRSLSLTRCPVTDRSLSMCLHKLQSLERLEISDCPELHDFPDDAMPMMASLKSLEFNGCHPLLMKKQQGRTGAAWERIRSIQRLEIV

SEQ ID NO: 13 - protein, 1154 aa, Oryza sativa
MATLPLATGVGWVVSPVIKLMFEKVQSYISTQYKWQSNLVDDLKKLETILTEILLVVGTAERRRTLDCNQQALLRQLKDAVYDAEDIMDEFDYMFLKANAQKRKLRSLGSSSISIAKRLVGHDKFRSKLGKMLKSLSAVKECAHMLVRVMGVENFSSHMLPEPLQWRISSSISIGEFVVGRQKEREELVHQLLEQSDKPESRSKGARSTSLEVITIVGNGGIGKTTLAQLIYNDKRIEDNFDMRAWVCVSHVFDKVRITKEILTTIDKSIDLTNFNFSMLQEELKNKITMKKFLLVLDDVWYDEKVGVPINADRWRELFAPLWHGAKVIKILVTTRMGIVANTLGCATPFCLSGLESKDSWELFRRCAFSTRDPNEHLELKSIGEHIVQKLNGSALAIKAVGGHLSSNFNYEEWNRVLKSGLSNEKDIMTILRLSYECLPEHLQQCFSFCGLFPKGYYFEPDMLVNMWIAHEFIQDRGRTYGSLTSTGKSYFDELLSRSFFQALRYGGTVHYVMHDLMNDLAVHVSNGKCYRVEANEPQEIFPEVQHRSILAERVDLLRACKLQRLRTLIIWNKERCYCSRVCVGVDFFKEFKSLRLLDLTGCCLRYLPDLNHMIHLRCLILPNTNRPLPDSLCSLYHLQMLFLHRHSCFICAKHVIFPKNLDNLSNILTIDVHRDLTVDLASVGHMPYLRAAGEFCVEKRKAQGLEVLHDMNELRGFLIFTSLENVKNKDEAIDAQLVNKSQISRLDLQWSFSNADSQSDKEYDVLNALTPHPCLEELNVEGYSGCTSPCWLESKWLSRLQHISIHDCTCWKLLPPLGQLPSLRELHIDGMKSLECIGTSFYGDAGFPSLKTLELTELPELADWSSIDYAFPVLHDVLISRCPKLKELPPVFPPPVKMEVLPSTIVYTQHTDHRLDTCITQKEVSLTSLSGIFHVCHQESVEIAEISFDGADMVNDGLRDLGPNLPSHQGPFICWYADFHRAFASLTEMKIVGCPNITSLLDFRYFPVLKNLIIQDCPELNELQEDGHLTTLTEVLIEHCNKLVSLRSLRNLFFLSKLEIRNCLKLVALPEMFGFFSLRVMIIHKCPEIVSLPEDGLPLTLNFLYLNGCHPLLEEQFEWQHGVEWEKYAMLPSCLFAGESIGYGQGNSKQLEF

SEQ ID NO: 14 - DNA, 3465 bp, Oryza sativa
  source 1..3465: mol_type = unassigned DNA
atggccactttaccactagccactggagttggatgggtagtatctcctgtcatcaagcttatgtttgagaaggtccaatcatatatatcaactcagtacaagtggcagtccaatttggtggatgaccttaaaaagctggagactattttaactgaaattctcttggtagtaggcactgcagaaaggcggagaacacttgattgcaatcagcaagctttactccgccagctgaaagatgctgtctacgatgccgaggacatcatggatgaatttgattacatgtttctgaaagcgaatgctcaaaagagaaagctaagaagcttaggctccagttctatctctattgccaagcgtttggttggccatgacaagtttcggtccaaattgggaaagatgctcaaaagcttgagtgcagtaaaggaatgtgcccatatgctcgtcagggtgatgggagtagaaaactttagttcacacatgttacctgagccccttcaatggcgtatctccagctcgatttcaattggtgagtttgtagttggtcgtcagaaggaacgggaagaactagtgcaccaattgctggaacaatctgacaaacctgaatctagaagcaaaggagcaaggtcaacatcattagaggtaattactatagtcggcaatggcggaattggaaaaactactttagctcaacttatttacaatgataaaagaatcgaggataattttgatatgagggcatgggtatgtgtatcacatgtctttgataaggtcagaatcaccaaagaaatcctaacaactattgataaaagcattgacctaacgaattttaattttagcatgctgcaagaagaactcaagaacaaaataaccatgaagaagtttctacttgtattggatgatgtttggtatgatgaaaaggttggggtacccataaatgctgatagatggagagaattgtttgctcctttatggcatggggcgaaagtaatcaagattttagttacaactcgaatgggtattgttgcaaatacattaggatgtgccactccattctgtttgagtggtctagagagtaaagatagctgggaacttttcagaagatgtgcatttagcactagagatccaaatgaacatctcgaattgaagtctataggtgaacacattgtgcaaaaattgaatggatcagcattagctataaaggctgttggtgggcatcttagttcaaacttcaactatgaagaatggaatcgagttctaaaaagtggtctatcgaatgagaaagatattatgacaattttacgcctaagctatgaatgcttgccagagcaccttcagcaatgcttttcgttctgtggtttgttcccaaaaggttattatttcgagcctgacatgttggttaacatgtggatagctcatgaatttattcaggatcgtggacgcacctatggaagcttaacaagcactgggaaaagttattttgatgagttgttatcaagatcatttttccaggcacttcgatatggaggtacagtgcattatgttatgcatgacctcatgaatgatcttgctgtccacgtgtccaatggtaagtgttacagagtagaagccaatgaacctcaagagatttttccagaagttcaacatcggtctatactggctgaaagagttgaccttcttcgtgcctgtaagttgcaaaggctgcgcaccctaataatttggaataaagaaagatgttattgctcacgagtttgtgtgggagtagattttttcaaagagttcaagagcttgagattattggatttgactggttgctgcttaagatatttgccggacttaaatcacatgatacaccttaggtgcttaattctcccaaatactaaccgtcctctacctgattcactctgcagtctttaccatttacaaatgttgtttctacaccggcattcatgttttatatgtgcaaaacatgtcatcttccccaaaaacctggataacctgagcaatattttgactattgatgttcatagggatcttactgttgatttggcttctgtggggcatatgccatacctccgggctgcaggggaattctgtgttgagaagaggaaagcgcaggggctagaggtgttgcatgacatgaatgaactccgagggtttcttatatttacatctctcgagaatgtgaaaaacaaggatgaagcaattgatgctcagttagtcaacaagagtcaaatatctaggttggacctacaatggagtttttctaatgcagatagccagtctgacaaagaatatgatgtgctcaatgctttaacacctcatccttgccttgaggaattgaatgttgaaggatactcaggctgtacatctccatgttggctggagtccaagtggctatctagattgcaacacatcagcattcatgattgcacatgttggaagttgcttccacctttaggtcagttaccatctctcagggaacttcatattgatggaatgaaatcattagagtgcatcggcacatctttctatggagatgctggctttccctccctgaaaacactagaattgacagaattgccagaattggcagattggtcttcaatcgattatgcttttcctgttcttcacgatgtactcatcagtaggtgtccaaagctgaaagaactgccaccagtctttcctccacctgtaaaaatggaagtgctcccatccaccatcgtttacacacagcatactgatcatcgcctggacacatgtattactcaaaaggaggttagcttaactagcctttcgggtatttttcacgtatgtcaccaggaatctgtggaaattgcagaaattagctttgacggagcagacatggtgaatgatgggcttagagatctaggccccaatcttccatcccaccaaggaccatttatctgctggtatgctgattttcaccgtgcgtttgcgagtttaacagaaatgaaaattgttggttgccccaacataacatcgttgttggacttcagatattttcctgtcctcaagaacttgatcatacaagattgccccgaattgaatgaactacaagaggatggacacctaacaaccttgacagaggttcttatagagcactgcaacaaactggtatcactgaggagcttgagaaacctttttttcctttccaaactggagatcagaaattgcctgaagttagtggctttgcctgagatgtttggcttcttctccctcagagtcatgatcatacacaaatgccctgaaattgtttctttaccggaagatggtcttcctctgacccttaactttttgtatttgaatggatgccatccattgctagaggagcagtttgaatggcaacatggtgttgagtgggagaagtatgccatgttgccgtcatgtttgtttgctggtgaatcgataggatatggtcaaggtaattcaaagcagcttgaattttga

SEQ ID NO: 15 - protein, 579 aa, Oryza sativa
MATLPLATGVGWVVSPVIKLMFEKVQSYISTQYKWQSNLVDDLKKLETILTEILLVVGTAERRRTLDCNQQALLRQLKDAVYDAEDIMDEFDYMFLKANAQKRKLRSLGSSSISIAKRLVGHDKFRSKLGKMLKSLSTVKECAHMLVRVMGVENFSSHMLPEPLQWRISSSISIGEFVVGRQKEREELVHQLLEQSDKPESRSKGARSTSLEVITIVGNGGIGKTTLAQLIYNDKRIEDNFDMRAWVCVSHVFDKVRITKEILTTIDKSIDLTNFNFSMLQEELKNKITMKKFLLVLDDVWYDEKVGVPINADRWRELFAPLWHGAKVIKILVTTRMGIVANTLGCATPFCLSGLESKDSWELFRRCAFSTRDPNEHLELKSIGEHIVQKLNGSALAIKAVGGHLSSNFNYEEWNRVLKSGLSNEKDIMTILRLSYECLPEHLQQCFSFCGLFPKGYYFEPDMLVNMWIAHEFIQDRGRTYGSLTSTGKSYFDELLSRSFFQALRYGGTVHYVMHDLMNDLAVHVSNGKCYRVEANEPQEIFPEVQHLSILAERVDLLRACKLQRLRTLIIWNKERCYC

SEQ ID NO: 16 - DNA, 1740 bp, Oryza sativa
  source 1..1740: mol_type = unassigned DNA
atggccactttaccactagccactggagttggatgggtagtatctcctgtcatcaagcttatgtttgagaaggtccaatcatatatatcaactcagtacaagtggcagtccaatttggtggatgaccttaaaaagctggagactattttaactgaaattctcttggtagtaggcactgcagaaaggcggagaacacttgattgcaatcagcaagctttactccgccagctgaaagatgctgtctacgatgccgaggacatcatggatgaatttgattacatgtttctgaaagcgaatgctcaaaagagaaagctaagaagcttaggctccagttctatctctattgccaagcgtttggttggccatgacaagtttcggtccaaattgggaaagatgctcaaaagcttgagtacagtaaaggaatgtgcccatatgctcgtcagggtgatgggagtagaaaactttagttcacacatgttacctgagccccttcaatggcgtatctccagctcgatttcaattggtgagtttgtagttggtcgtcagaaggaacgggaagaactagtgcaccaattgctggaacaatctgacaaacctgaatctagaagcaaaggagcaaggtcaacatcattagaggtaattactatagtcggcaatggcggaattggaaaaactactttagctcaacttatttacaatgataaaagaatcgaggataattttgatatgagggcatgggtatgtgtatcacatgtctttgataaggtcagaatcaccaaagaaatcctaacaactattgataaaagcattgacctaacgaattttaattttagcatgctgcaagaagaactcaagaacaaaataaccatgaagaagtttctacttgtattggatgatgtttggtatgatgaaaaggttggggtacccataaatgctgatagatggagagaattgtttgctcctttatggcatggggcgaaagtaatcaagattttagttacaactcgaatgggtattgttgcaaatacattaggatgtgccactccattctgtttgagtggtctagagagtaaagatagctgggaacttttcagaagatgtgcatttagcactagagatccaaatgaacatctcgaattgaagtctataggtgaacacattgtgcaaaaattgaatggatcggcattagctataaaggctgttggtgggcatcttagttcaaacttcaactatgaagaatggaatcgagttctaaaaagtggtctatcgaatgagaaagatattatgacaattttacgcctaagctatgaatgcttgccagagcaccttcagcaatgcttttcgttctgtggtttgttcccaaaaggttattatttcgagcctgacatgttggttaacatgtggatagctcatgaatttattcaggatcgtggacgcacctatggaagcttgacaagcactgggaaaagttattttgatgagttgttatcaagatcatttttccaggcacttcgatatggaggtacagtgcattatgttatgcatgacctcatgaatgatcttgctgtccacgtgtccaatggtaagtgttacagagtagaagccaatgaacctcaagagatttttccagaagttcaacatctgtctatactggctgaaagagttgaccttcttcgtgcctgtaagttgcaaaggctgcgcaccctaataatttggaataaagaaagatgttattgctaa